European Patent Application EP 4 450 626 A1, published October 23, 2024. Title: FNIP2 INHIBITORS FOR TREATING ATAXIA TELANGIECTASIA. Applicant: IFOM - Istituto Fondazione di Oncologia Molecolare ETS. Application EP. The sequence listing filed with the application follows.

SEQUENCE LISTING (11 sequences)

SEQ ID NO: 1 - DNA, 16 bp, synthetic construct
  source 1..16: mol_type = other DNA
  modified_base 1..4: mod_base = OTHER; note = locked nucleic acid
  modified_base 13..16: mod_base = OTHER; note = locked nucleic acid
agtaggtcaggacata

SEQ ID NO: 2 - DNA, 16 bp, synthetic construct
  source 1..16: mol_type = other DNA
  modified_base 1..4: mod_base = OTHER; note = locked nucleic acid
  modified_base 13..16: mod_base = OTHER; note = locked nucleic acid
gaaagtaggtcaggac

SEQ ID NO: 3 - DNA, 16 bp, synthetic construct
  source 1..16: mol_type = other DNA
  modified_base 1..4: mod_base = OTHER; note = locked nucleic acid
  modified_base 13..16: mod_base = OTHER; note = locked nucleic acid
gtggaggagaacgtat

SEQ ID NO: 4 - DNA, 16 bp, synthetic construct
  source 1..16: mol_type = other DNA
  modified_base 1..4: mod_base = OTHER; note = locked nucleic acid
  modified_base 13..16: mod_base = OTHER; note = locked nucleic acid
acggctgacataaaac

SEQ ID NO: 5 - DNA, 16 bp, synthetic construct
  source 1..16: mol_type = other DNA
  modified_base 1..4: mod_base = OTHER; note = locked nucleic acid
  modified_base 13..16: mod_base = OTHER; note = locked nucleic acid
cgattctgaggacagc

SEQ ID NO: 6 - DNA, 29 bp, synthetic construct
  source 1..29: mol_type = other DNA
tcggagtttgacctgaatgagattcgcct

SEQ ID NO: 7 - DNA, 29 bp, synthetic construct
  source 1..29: mol_type = other DNA
ccaagaaggtcaactgatgagacattcag

SEQ ID NO: 8 - DNA, 29 bp, synthetic construct
  source 1..29: mol_type = other DNA
gctgttgaaagtggagatgcctacaagac

SEQ ID NO: 9 - DNA, 29 bp, synthetic construct
  source 1..29: mol_type = other DNA
aacgacctgcctctgttgactgctattgc

SEQ ID NO: 10 - DNA, 22 bp, synthetic construct
  source 1..22: mol_type = other DNA
ctttgtcaagctcatttcctgg

SEQ ID NO: 11 - DNA, 19 bp, synthetic construct
  source 1..19: mol_type = other DNA
tcttgctcagtgtccttgc